European Patent Application EP 4 174 091 A1, published May 3, 2023. Title: ANTI-CD44 SINGLE-CHAIN ANTIBODY AND USE THEREOF IN PREPARING DRUG FOR TREATING TUMOR. Applicant: Beijing Neurosurgical Institute. The sequence listing filed with the application follows.

SEQUENCE LISTING (14 sequences)

SEQ ID NO: 1 - protein, 246 aa, Artificial Sequence
  This sequence is synthesized in lab.
QVQLVESGGGVVQPGRSLRLSCAASGFTFSSYGMHWVRQAPGKGLEWVAVIWYDGSNKFYADSVKGRFTISRDNSKNTLYLQMNSLRAEDTAVYYCARRSDYRGYYGMDVWGQGTTVTVSSGSTSGGGSGGGSGGGGSSEIVLTQSPATLSLSPGERATLSCRASQSVINYLAWYQQKPGQAPRLLIYDASNRASGIPARFSGSGSGTDFTLTISSLEPEDFAVYYCQQRRNWPLTFGGGTKVEIK

SEQ ID NO: 2 - DNA, 738 bp, Artificial Sequence
  This sequence is synthesized in lab.
caggtgcagctggtggagtctgggggaggcgtggtccagcctgggaggtccctgagactctcctgtgcagcgtctggattcaccttcagtagctatggcatgcactgggtccgccaggctccaggcaaggggctggagtgggtggcagttatatggtatgatggaagtaataaattctatgcagactccgtgaagggccgattcaccatctccagagacaattccaagaacacgctgtatctgcaaatgaacagcctgagagccgaggacacggctgtgtattactgtgcgaggagaagtgactacaggggctactacggtatggacgtctggggccaagggaccacggtcaccgtctcctcaggcagtactagcggtggtggctccgggggcggttccggtgggggcggcagcagcgaaattgtgttgacacagtctccagccaccctgtctttgtctccaggggaaagagccaccctctcctgcagggccagtcagagtgttatcaactacttagcctggtaccaacagaaacctggccaggctcccaggctcctcatctatgatgcatccaacagggcctctggcatcccagccaggttcagtggcagtgggtctgggacagacttcactctcaccatcagcagcctagagcctgaagattttgcagtttattactgtcagcagcgtcgcaactggccgctcactttcggcggagggaccaaggtggagatcaaa

SEQ ID NO: 3 - protein, 468 aa, Artificial Sequence
  This sequence is synthesized in lab.
QVQLVESGGGVVQPGRSLRLSCAASGFTFSSYGMHWVRQAPGKGLEWVAVIWYDGSNKFYADSVKGRFTISRDNSKNTLYLQMNSLRAEDTAVYYCARRSDYRGYYGMDVWGQGTTVTVSSGSTSGGGSGGGSGGGGSSEIVLTQSPATLSLSPGERATLSCRASQSVINYLAWYQQKPGQAPRLLIYDASNRASGIPARFSGSGSGTDFTLTISSLEPEDFAVYYCQQRRNWPLTFGGGTKVEIKTTTPAPRPPTPAPTIASQPLSLRPEACRPAAGGAVHTRGLDFACDIYIWAPLAGTCGVLLLSLVITLYCRSKRSRLLHSDYMNMTPRRPGPTRKHYQPYAPPRDFAAYRSRVKFSRSADAPAYKQGQNQLYNELNLGRREEYDVLDKRRGRDPEMGGKPRRKNPQEGLYNELQKDKMAEAYSEIGMKGERRRGKGHDGLYQGLSTATKDTYDALHMQALPPR

SEQ ID NO: 4 - protein, 727 aa, Artificial Sequence
  This sequence is synthesized in lab.
QVQLVESGGGVVQPGRSLRLSCAASGFTFSSYGMHWVRQAPGKGLEWVAVIWYDGSNKFYADSVKGRFTISRDNSKNTLYLQMNSLRAEDTAVYYCARRSDYRGYYGMDVWGQGTTVTVSSGSTSGGGSGGGSGGGGSSEIVLTQSPATLSLSPGERATLSCRASQSVINYLAWYQQKPGQAPRLLIYDASNRASGIPARFSGSGSGTDFTLTISSLEPEDFAVYYCQQRRNWPLTFGGGTKVEIKGGGGSGGGGSGGGGSQVQLVQSGAEVKKPGASVKVSCKASGYTFTDFEMHWVRQAPGQGLEWMGDIDPGTGDTAYNLKFKGRVTMTTDTSTSTAYMELRSLRSDDTAVYYCALGAFVYWGQGTLVTVSSGSTSGGGSGGGSGGGGSSDVVMTQSPLSLPVTPGEPASISCRSSQSLANSYGNTYLSWYLQKPGQSPQLLIYGISNRFSGVPDRFSGSGSGTDFTLKISRVEAEDVGVYYCLQGTHQPYTFGQGTKLEIKTTTPAPRPPTPAPTIASQPLSLRPEACRPAAGGAVHTRGLDFACDIYIWAPLAGTCGVLLLSLVITLYCRSKRSRLLHSDYMNMTPRRPGPTRKHYQPYAPPRDFAAYRSRVKFSRSADAPAYKQGQNQLYNELNLGRREEYDVLDKRRGRDPEMGGKPRRKNPQEGLYNELQKDKMAEAYSEIGMKGERRRGKGHDGLYQGLSTATKDTYDALHMQALPPR

SEQ ID NO: 5 - protein, 563 aa, Artificial Sequence
  This sequence is synthesized in lab.
QVQLVESGGGVVQPGRSLRLSCAASGFTFSSYGMHWVRQAPGKGLEWVAVIWYDGSNKFYADSVKGRFTISRDNSKNTLYLQMNSLRAEDTAVYYCARRSDYRGYYGMDVWGQGTTVTVSSGSTSGGGSGGGSGGGGSSEIVLTQSPATLSLSPGERATLSCRASQSVINYLAWYQQKPGQAPRLLIYDASNRASGIPARFSGSGSGTDFTLTISSLEPEDFAVYYCQQRRNWPLTFGGGTKVEIKTTTPAPRPPTPAPTIASQPLSLRPEACRPAAGGAVHTRGLDFACDIYIWAPLAGTCGVLLLSLVITLYCRSKRSRLLHSDYMNMTPRRPGPTRKHYQPYAPPRDFAAYRSKKRIKPIVWPSLPDHKKTLEHLCKKPRKNLNVSFNPESFLDCQIHRVDDIQARDEVEGFLQDTFPQQLEESEKQRLLGSNQEEAYVTMSSFYQNQRVKFSRSADAPAYKQGQNQLYNELNLGRREEYDVLDKRRGRDPEMGGKPRRKNPQEGLYNELQKDKMAEAYSEIGMKGERRRGKGHDGLYQGLSTATKDTYDALHMQALPPR

SEQ ID NO: 6 - protein, 739 aa, Artificial Sequence
  This sequence is synthesized in lab.
QVQLVESGGGVVQPGRSLRLSCAASGFTFSSYGMHWVRQAPGKGLEWVAVIWYDGSNKFYADSVKGRFTISRDNSKNTLYLQMNSLRAEDTAVYYCARRSDYRGYYGMDVWGQGTTVTVSSGSTSGGGSGGGSGGGGSSEIVLTQSPATLSLSPGERATLSCRASQSVINYLAWYQQKPGQAPRLLIYDASNRASGIPARFSGSGSGTDFTLTISSLEPEDFAVYYCQQRRNWPLTFGGGTKVEIKTTTPAPRPPTPAPTIASQPLSLRPEACRPAAGGAVHTRGLDFACDIYIWAPLAGTCGVLLLSLVITLYCRSKRSRLLHSDYMNMTPRRPGPTRKHYQPYAPPRDFAAYRSRVKFSRSADAPAYKQGQNQLYNELNLGRREEYDVLDKRRGRDPEMGGKPRRKNPQEGLYNELQKDKMAEAYSEIGMKGERRRGKGHDGLYQGLSTATKDTYDALHMQALPPREGRGSLLTCGDVEENPGPMTNKCLLQIALLLCFSTTALSQVQLQQSGPGLVKPSHTLSLTCTVSGGSISSGGYYWSWTRQHPGMGLEWIGYISYSGSIYYTPSLKSRLTISVDTSKNQFSLKLSSVTAADTAVYYCASLDSWGSNRDYWGQGTLVTVSSGGGGSEIVLTQSPATLSLSPGERATLSCRASQSVSSYLAWYQQKPGQAPRLLIYDASNRATGIPARFSGSGSGTDFTLTISSLEPEDFAVYYCQQRSNWPLTFGGGTKVEIK

SEQ ID NO: 7 - protein, 834 aa, Artificial Sequence
  This sequence is synthesized in lab.
QVQLVESGGGVVQPGRSLRLSCAASGFTFSSYGMHWVRQAPGKGLEWVAVIWYDGSNKFYADSVKGRFTISRDNSKNTLYLQMNSLRAEDTAVYYCARRSDYRGYYGMDVWGQGTTVTVSSGSTSGGGSGGGSGGGGSSEIVLTQSPATLSLSPGERATLSCRASQSVINYLAWYQQKPGQAPRLLIYDASNRASGIPARFSGSGSGTDFTLTISSLEPEDFAVYYCQQRRNWPLTFGGGTKVEIKTTTPAPRPPTPAPTIASQPLSLRPEACRPAAGGAVHTRGLDFACDIYIWAPLAGTCGVLLLSLVITLYCRSKRSRLLHSDYMNMTPRRPGPTRKHYQPYAPPRDFAAYRSKKRIKPIVWPSLPDHKKTLEHLCKKPRKNLNVSFNPESFLDCQIHRVDDIQARDEVEGFLQDTFPQQLEESEKQRLLGSNQEEAYVTMSSFYQNQRVKFSRSADAPAYKQGQNQLYNELNLGRREEYDVLDKRRGRDPEMGGKPRRKNPQEGLYNELQKDKMAEAYSEIGMKGERRRGKGHDGLYQGLSTATKDTYDALHMQALPPREGRGSLLTCGDVEENPGPMTNKCLLQIALLLCFSTTALSQVQLQQSGPGLVKPSHTLSLTCTVSGGSISSGGYYWSWTRQHPGMGLEWIGYISYSGSIYYTPSLKSRLTISVDTSKNQFSLKLSSVTAADTAVYYCASLDSWGSNRDYWGQGTLVTVSSGGGGSEIVLTQSPATLSLSPGERATLSCRASQSVSSYLAWYQQKPGQAPRLLIYDASNRATGIPARFSGSGSGTDFTLTISSLEPEDFAVYYCQQRSNWPLTFGGGTKVEIK

SEQ ID NO: 8 - protein, 1093 aa, Artificial Sequence
  This sequence is synthesized in lab.
QVQLVESGGGVVQPGRSLRLSCAASGFTFSSYGMHWVRQAPGKGLEWVAVIWYDGSNKFYADSVKGRFTISRDNSKNTLYLQMNSLRAEDTAVYYCARRSDYRGYYGMDVWGQGTTVTVSSGSTSGGGSGGGSGGGGSSEIVLTQSPATLSLSPGERATLSCRASQSVINYLAWYQQKPGQAPRLLIYDASNRASGIPARFSGSGSGTDFTLTISSLEPEDFAVYYCQQRRNWPLTFGGGTKVEIKGGGGSGGGGSGGGGSQVQLVQSGAEVKKPGASVKVSCKASGYTFTDFEMHWVRQAPGQGLEWMGDIDPGTGDTAYNLKFKGRVTMTTDTSTSTAYMELRSLRSDDTAVYYCALGAFVYWGQGTLVTVSSGSTSGGGSGGGSGGGGSSDVVMTQSPLSLPVTPGEPASISCRSSQSLANSYGNTYLSWYLQKPGQSPQLLIYGISNRFSGVPDRFSGSGSGTDFTLKISRVEAEDVGVYYCLQGTHQPYTFGQGTKLEIKTTTPAPRPPTPAPTIASQPLSLRPEACRPAAGGAVHTRGLDFACDIYIWAPLAGTCGVLLLSLVITLYCRSKRSRLLHSDYMNMTPRRPGPTRKHYQPYAPPRDFAAYRSKKRIKPIVWPSLPDHKKTLEHLCKKPRKNLNVSFNPESFLDCQIHRVDDIQARDEVEGFLQDTFPQQLEESEKQRLLGSNQEEAYVTMSSFYQNQRVKFSRSADAPAYKQGQNQLYNELNLGRREEYDVLDKRRGRDPEMGGKPRRKNPQEGLYNELQKDKMAEAYSEIGMKGERRRGKGHDGLYQGLSTATKDTYDALHMQALPPREGRGSLLTCGDVEENPGPMTNKCLLQIALLLCFSTTALSQVQLQQSGPGLVKPSHTLSLTCTVSGGSISSGGYYWSWTRQHPGMGLEWIGYISYSGSIYYTPSLKSRLTISVDTSKNQFSLKLSSVTAADTAVYYCASLDSWGSNRDYWGQGTLVTVSSGGGGSEIVLTQSPATLSLSPGERATLSCRASQSVSSYLAWYQQKPGQAPRLLIYDASNRATGIPARFSGSGSGTDFTLTISSLEPEDFAVYYCQQRSNWPLTFGGGTKVEIK

SEQ ID NO: 9 - DNA, 1404 bp, Artificial Sequence
  This sequence is synthesized in lab.
caggtgcagctggtggagtctgggggaggcgtggtccagcctgggaggtccctgagactctcctgtgcagcgtctggattcaccttcagtagctatggcatgcactgggtccgccaggctccaggcaaggggctggagtgggtggcagttatatggtatgatggaagtaataaattctatgcagactccgtgaagggccgattcaccatctccagagacaattccaagaacacgctgtatctgcaaatgaacagcctgagagccgaggacacggctgtgtattactgtgcgaggagaagtgactacaggggctactacggtatggacgtctggggccaagggaccacggtcaccgtctcctcaggcagtactagcggtggtggctccgggggcggttccggtgggggcggcagcagcgaaattgtgttgacacagtctccagccaccctgtctttgtctccaggggaaagagccaccctctcctgcagggccagtcagagtgttatcaactacttagcctggtaccaacagaaacctggccaggctcccaggctcctcatctatgatgcatccaacagggcctctggcatcccagccaggttcagtggcagtgggtctgggacagacttcactctcaccatcagcagcctagagcctgaagattttgcagtttattactgtcagcagcgtcgcaactggccgctcactttcggcggagggaccaaggtggagatcaaaaccactaccccagcaccgaggccacccaccccggctcctaccatcgcctcccagcctctgtccctgcgtccggaggcatgtagacccgcagctggtggggccgtgcatacccggggtcttgacttcgcctgcgatatctacatttgggcccctctggctggtacttgcggggtcctgctgctttcactcgtgatcactctttactgtaggagtaagaggagcaggctcctgcacagtgactacatgaacatgactccccgccgccccgggcccacccgcaagcattaccagccctatgccccaccacgcgacttcgcagcctatcgctcccgcgtgaaattcagccgcagcgcagatgctccagcctacaagcaggggcagaaccagctctacaacgaactcaatcttggtcggagagaggagtacgacgtgctggacaagcggagaggacgggacccagaaatgggcgggaagccgcgcagaaagaatccccaagagggcctgtacaacgagctccaaaaggataagatggcagaagcctatagcgagattggtatgaaaggggaacgcagaagaggcaaaggccacgacggactgtaccagggactcagcaccgccaccaaggacacctatgacgctcttcacatgcaggccctgccgcctcgg

SEQ ID NO: 10 - DNA, 2181 bp, Artificial Sequence
  This sequence is synthesized in lab.
caggtgcagctggtggagtctgggggaggcgtggtccagcctgggaggtccctgagactctcctgtgcagcgtctggattcaccttcagtagctatggcatgcactgggtccgccaggctccaggcaaggggctggagtgggtggcagttatatggtatgatggaagtaataaattctatgcagactccgtgaagggccgattcaccatctccagagacaattccaagaacacgctgtatctgcaaatgaacagcctgagagccgaggacacggctgtgtattactgtgcgaggagaagtgactacaggggctactacggtatggacgtctggggccaagggaccacggtcaccgtctcctcaggcagtactagcggtggtggctccgggggcggttccggtgggggcggcagcagcgaaattgtgttgacacagtctccagccaccctgtctttgtctccaggggaaagagccaccctctcctgcagggccagtcagagtgttatcaactacttagcctggtaccaacagaaacctggccaggctcccaggctcctcatctatgatgcatccaacagggcctctggcatcccagccaggttcagtggcagtgggtctgggacagacttcactctcaccatcagcagcctagagcctgaagattttgcagtttattactgtcagcagcgtcgcaactggccgctcactttcggcggagggaccaaggtggagatcaaaggaggtggtggatccggaggtggtggctccggaggtggtggatcccaggttcagctggtgcagtctggagctgaggtgaagaagcctggggcctcagtgaaggtctcctgcaaggcttctggttacacctttaccgactttgaaatgcactgggtgcgacaggcccctggacaagggcttgagtggatgggagatattgatcctggaactggtgatactgcctacaatctgaagttcaagggcagagtcaccatgaccacagacacatccacgagcacagcctacatggagctgaggagcctgaggtctgacgacacggccgtgtattactgtgcgttgggggcctttgtttactggggccagggaaccctggtcaccgtctcctcaggcagtactagcggtggtggctccgggggcggttccggtgggggcggcagcagcgatgttgtgatgactcagtctccactctccctgcccgtcacccctggagagccggcctccatctcctgcaggtctagtcagagtcttgcaaacagttatgggaacacctatttgtcttggtacctgcagaagccagggcagtctccacagctcctgatctatgggatttccaacagattttctggggtccctgacaggttcagtggcagtggatcaggcacagattttacactgaaaatcagcagagtggaggctgaggacgttggggtttattactgcttacaaggtacacatcagccgtacacgtttggccaggggaccaagctggagatcaaaaccactaccccagcaccgaggccacccaccccggctcctaccatcgcctcccagcctctgtccctgcgtccggaggcatgtagacccgcagctggtggggccgtgcatacccggggtcttgacttcgcctgcgatatctacatttgggcccctctggctggtacttgcggggtcctgctgctttcactcgtgatcactctttactgtaggagtaagaggagcaggctcctgcacagtgactacatgaacatgactccccgccgccccgggcccacccgcaagcattaccagccctatgccccaccacgcgacttcgcagcctatcgctcccgcgtgaaattcagccgcagcgcagatgctccagcctacaagcaggggcagaaccagctctacaacgaactcaatcttggtcggagagaggagtacgacgtgctggacaagcggagaggacgggacccagaaatgggcgggaagccgcgcagaaagaatccccaagagggcctgtacaacgagctccaaaaggataagatggcagaagcctatagcgagattggtatgaaaggggaacgcagaagaggcaaaggccacgacggactgtaccagggactcagcaccgccaccaaggacacctatgacgctcttcacatgcaggccctgccgcctcgg

SEQ ID NO: 11 - DNA, 1689 bp, Artificial Sequence
  This sequence is synthesized in lab.
caggtgcagctggtggagtctgggggaggcgtggtccagcctgggaggtccctgagactctcctgtgcagcgtctggattcaccttcagtagctatggcatgcactgggtccgccaggctccaggcaaggggctggagtgggtggcagttatatggtatgatggaagtaataaattctatgcagactccgtgaagggccgattcaccatctccagagacaattccaagaacacgctgtatctgcaaatgaacagcctgagagccgaggacacggctgtgtattactgtgcgaggagaagtgactacaggggctactacggtatggacgtctggggccaagggaccacggtcaccgtctcctcaggcagtactagcggtggtggctccgggggcggttccggtgggggcggcagcagcgaaattgtgttgacacagtctccagccaccctgtctttgtctccaggggaaagagccaccctctcctgcagggccagtcagagtgttatcaactacttagcctggtaccaacagaaacctggccaggctcccaggctcctcatctatgatgcatccaacagggcctctggcatcccagccaggttcagtggcagtgggtctgggacagacttcactctcaccatcagcagcctagagcctgaagattttgcagtttattactgtcagcagcgtcgcaactggccgctcactttcggcggagggaccaaggtggagatcaaaaccactaccccagcaccgaggccacccaccccggctcctaccatcgcctcccagcctctgtccctgcgtccggaggcatgtagacccgcagctggtggggccgtgcatacccggggtcttgacttcgcctgcgatatctacatttgggcccctctggctggtacttgcggggtcctgctgctttcactcgtgatcactctttactgtaggagtaagaggagcaggctcctgcacagtgactacatgaacatgactccccgccgccccgggcccacccgcaagcattaccagccctatgccccaccacgcgacttcgcagcctatcgctccaaaaaaaggattaagcctatcgtatggcccagtctccccgatcacaagaagactctggaacacctttgtaagaaaccaagaaaaaatttaaatgtgagtttcaatcctgaaagtttcctggactgccagattcatagggtggatgacattcaagctagagatgaagtggaaggttttctgcaagatacgtttcctcagcaactagaagaatctgagaagcagaggcttctgggatcaaatcaagaagaagcatatgtcaccatgtccagcttctaccaaaaccagcgcgtgaaattcagccgcagcgcagatgctccagcctacaagcaggggcagaaccagctctacaacgaactcaatcttggtcggagagaggagtacgacgtgctggacaagcggagaggacgggacccagaaatgggcgggaagccgcgcagaaagaatccccaagagggcctgtacaacgagctccaaaaggataagatggcagaagcctatagcgagattggtatgaaaggggaacgcagaagaggcaaaggccacgacggactgtaccagggactcagcaccgccaccaaggacacctatgacgctcttcacatgcaggccctgccgcctcgg

SEQ ID NO: 12 - DNA, 2217 bp, Artificial Sequence
  This sequence is synthesized in lab.
caggtgcagctggtggagtctgggggaggcgtggtccagcctgggaggtccctgagactctcctgtgcagcgtctggattcaccttcagtagctatggcatgcactgggtccgccaggctccaggcaaggggctggagtgggtggcagttatatggtatgatggaagtaataaattctatgcagactccgtgaagggccgattcaccatctccagagacaattccaagaacacgctgtatctgcaaatgaacagcctgagagccgaggacacggctgtgtattactgtgcgaggagaagtgactacaggggctactacggtatggacgtctggggccaagggaccacggtcaccgtctcctcaggcagtactagcggtggtggctccgggggcggttccggtgggggcggcagcagcgaaattgtgttgacacagtctccagccaccctgtctttgtctccaggggaaagagccaccctctcctgcagggccagtcagagtgttatcaactacttagcctggtaccaacagaaacctggccaggctcccaggctcctcatctatgatgcatccaacagggcctctggcatcccagccaggttcagtggcagtgggtctgggacagacttcactctcaccatcagcagcctagagcctgaagattttgcagtttattactgtcagcagcgtcgcaactggccgctcactttcggcggagggaccaaggtggagatcaaaaccactaccccagcaccgaggccacccaccccggctcctaccatcgcctcccagcctctgtccctgcgtccggaggcatgtagacccgcagctggtggggccgtgcatacccggggtcttgacttcgcctgcgatatctacatttgggcccctctggctggtacttgcggggtcctgctgctttcactcgtgatcactctttactgtaggagtaagaggagcaggctcctgcacagtgactacatgaacatgactccccgccgccccgggcccacccgcaagcattaccagccctatgccccaccacgcgacttcgcagcctatcgctcccgcgtgaaattcagccgcagcgcagatgctccagcctacaagcaggggcagaaccagctctacaacgaactcaatcttggtcggagagaggagtacgacgtgctggacaagcggagaggacgggacccagaaatgggcgggaagccgcgcagaaagaatccccaagagggcctgtacaacgagctccaaaaggataagatggcagaagcctatagcgagattggtatgaaaggggaacgcagaagaggcaaaggccacgacggactgtaccagggactcagcaccgccaccaaggacacctatgacgctcttcacatgcaggccctgccgcctcgggagggaaggggttctctcctgacctgcggcgatgtggaggagaaccccggacccatgaccaacaagtgtctcctccaaattgctctcctgttgtgcttctccactacagctctttcccaggtgcagctacagcagtcgggcccaggactggtgaagccttcacacaccctgtccctcacctgcactgtctctggtggctccatcagcagtggtggttactactggagttggacccgtcagcacccagggatgggcctggagtggattggatacatctcttacagtgggagtatctattacactccgtccctcaagagtcgacttaccatatcagtggacacgtctaagaaccagttctccctgaagctgagctctgtgactgccgcggacacggccgtatattactgtgcgagtttggattcctggggatctaaccgtgactactggggccagggaaccctggtcaccgtctcgagtggaggtggtggatccgaaattgtgttgacgcagtctccagccaccctgtctttgtctccaggggaaagagccaccctctcctgcagggccagtcagagtgttagcagctacttagcctggtaccaacagaaacctggccaggctcccaggctcctcatctatgatgcatccaacagggccactggcatcccagccaggttcagtggcagtgggtctgggacagacttcactctcaccatcagcagcctagagcctgaagattttgcagtttattactgtcagcagcgtagcaactggccgctcactttcggcggagggaccaaggtggagattaag

SEQ ID NO: 13 - DNA, 2502 bp, Artificial Sequence
  This sequence is synthesized in lab.
caggtgcagctggtggagtctgggggaggcgtggtccagcctgggaggtccctgagactctcctgtgcagcgtctggattcaccttcagtagctatggcatgcactgggtccgccaggctccaggcaaggggctggagtgggtggcagttatatggtatgatggaagtaataaattctatgcagactccgtgaagggccgattcaccatctccagagacaattccaagaacacgctgtatctgcaaatgaacagcctgagagccgaggacacggctgtgtattactgtgcgaggagaagtgactacaggggctactacggtatggacgtctggggccaagggaccacggtcaccgtctcctcaggcagtactagcggtggtggctccgggggcggttccggtgggggcggcagcagcgaaattgtgttgacacagtctccagccaccctgtctttgtctccaggggaaagagccaccctctcctgcagggccagtcagagtgttatcaactacttagcctggtaccaacagaaacctggccaggctcccaggctcctcatctatgatgcatccaacagggcctctggcatcccagccaggttcagtggcagtgggtctgggacagacttcactctcaccatcagcagcctagagcctgaagattttgcagtttattactgtcagcagcgtcgcaactggccgctcactttcggcggagggaccaaggtggagatcaaaaccactaccccagcaccgaggccacccaccccggctcctaccatcgcctcccagcctctgtccctgcgtccggaggcatgtagacccgcagctggtggggccgtgcatacccggggtcttgacttcgcctgcgatatctacatttgggcccctctggctggtacttgcggggtcctgctgctttcactcgtgatcactctttactgtaggagtaagaggagcaggctcctgcacagtgactacatgaacatgactccccgccgccccgggcccacccgcaagcattaccagccctatgccccaccacgcgacttcgcagcctatcgctccaaaaaaaggattaagcctatcgtatggcccagtctccccgatcacaagaagactctggaacacctttgtaagaaaccaagaaaaaatttaaatgtgagtttcaatcctgaaagtttcctggactgccagattcatagggtggatgacattcaagctagagatgaagtggaaggttttctgcaagatacgtttcctcagcaactagaagaatctgagaagcagaggcttctgggatcaaatcaagaagaagcatatgtcaccatgtccagcttctaccaaaaccagcgcgtgaaattcagccgcagcgcagatgctccagcctacaagcaggggcagaaccagctctacaacgaactcaatcttggtcggagagaggagtacgacgtgctggacaagcggagaggacgggacccagaaatgggcgggaagccgcgcagaaagaatccccaagagggcctgtacaacgagctccaaaaggataagatggcagaagcctatagcgagattggtatgaaaggggaacgcagaagaggcaaaggccacgacggactgtaccagggactcagcaccgccaccaaggacacctatgacgctcttcacatgcaggccctgccgcctcgggagggaaggggttctctcctgacctgcggcgatgtggaggagaaccccggacccatgaccaacaagtgtctcctccaaattgctctcctgttgtgcttctccactacagctctttcccaggtgcagctacagcagtcgggcccaggactggtgaagccttcacacaccctgtccctcacctgcactgtctctggtggctccatcagcagtggtggttactactggagttggacccgtcagcacccagggatgggcctggagtggattggatacatctcttacagtgggagtatctattacactccgtccctcaagagtcgacttaccatatcagtggacacgtctaagaaccagttctccctgaagctgagctctgtgactgccgcggacacggccgtatattactgtgcgagtttggattcctggggatctaaccgtgactactggggccagggaaccctggtcaccgtctcgagtggaggtggtggatccgaaattgtgttgacgcagtctccagccaccctgtctttgtctccaggggaaagagccaccctctcctgcagggccagtcagagtgttagcagctacttagcctggtaccaacagaaacctggccaggctcccaggctcctcatctatgatgcatccaacagggccactggcatcccagccaggttcagtggcagtgggtctgggacagacttcactctcaccatcagcagcctagagcctgaagattttgcagtttattactgtcagcagcgtagcaactggccgctcactttcggcggagggaccaaggtggagattaag

SEQ ID NO: 14 - DNA, 3279 bp, Artificial Sequence
  This sequence is synthesized in lab.
caggtgcagctggtggagtctgggggaggcgtggtccagcctgggaggtccctgagactctcctgtgcagcgtctggattcaccttcagtagctatggcatgcactgggtccgccaggctccaggcaaggggctggagtgggtggcagttatatggtatgatggaagtaataaattctatgcagactccgtgaagggccgattcaccatctccagagacaattccaagaacacgctgtatctgcaaatgaacagcctgagagccgaggacacggctgtgtattactgtgcgaggagaagtgactacaggggctactacggtatggacgtctggggccaagggaccacggtcaccgtctcctcaggcagtactagcggtggtggctccgggggcggttccggtgggggcggcagcagcgaaattgtgttgacacagtctccagccaccctgtctttgtctccaggggaaagagccaccctctcctgcagggccagtcagagtgttatcaactacttagcctggtaccaacagaaacctggccaggctcccaggctcctcatctatgatgcatccaacagggcctctggcatcccagccaggttcagtggcagtgggtctgggacagacttcactctcaccatcagcagcctagagcctgaagattttgcagtttattactgtcagcagcgtcgcaactggccgctcactttcggcggagggaccaaggtggagatcaaaggaggtggtggatccggaggtggtggctccggaggtggtggatcccaggttcagctggtgcagtctggagctgaggtgaagaagcctggggcctcagtgaaggtctcctgcaaggcttctggttacacctttaccgactttgaaatgcactgggtgcgacaggcccctggacaagggcttgagtggatgggagatattgatcctggaactggtgatactgcctacaatctgaagttcaagggcagagtcaccatgaccacagacacatccacgagcacagcctacatggagctgaggagcctgaggtctgacgacacggccgtgtattactgtgcgttgggggcctttgtttactggggccagggaaccctggtcaccgtctcctcaggcagtactagcggtggtggctccgggggcggttccggtgggggcggcagcagcgatgttgtgatgactcagtctccactctccctgcccgtcacccctggagagccggcctccatctcctgcaggtctagtcagagtcttgcaaacagttatgggaacacctatttgtcttggtacctgcagaagccagggcagtctccacagctcctgatctatgggatttccaacagattttctggggtccctgacaggttcagtggcagtggatcaggcacagattttacactgaaaatcagcagagtggaggctgaggacgttggggtttattactgcttacaaggtacacatcagccgtacacgtttggccaggggaccaagctggagatcaaaaccactaccccagcaccgaggccacccaccccggctcctaccatcgcctcccagcctctgtccctgcgtccggaggcatgtagacccgcagctggtggggccgtgcatacccggggtcttgacttcgcctgcgatatctacatttgggcccctctggctggtacttgcggggtcctgctgctttcactcgtgatcactctttactgtaggagtaagaggagcaggctcctgcacagtgactacatgaacatgactccccgccgccccgggcccacccgcaagcattaccagccctatgccccaccacgcgacttcgcagcctatcgctccaaaaaaaggattaagcctatcgtatggcccagtctccccgatcacaagaagactctggaacacctttgtaagaaaccaagaaaaaatttaaatgtgagtttcaatcctgaaagtttcctggactgccagattcatagggtggatgacattcaagctagagatgaagtggaaggttttctgcaagatacgtttcctcagcaactagaagaatctgagaagcagaggcttctgggatcaaatcaagaagaagcatatgtcaccatgtccagcttctaccaaaaccagcgcgtgaaattcagccgcagcgcagatgctccagcctacaagcaggggcagaaccagctctacaacgaactcaatcttggtcggagagaggagtacgacgtgctggacaagcggagaggacgggacccagaaatgggcgggaagccgcgcagaaagaatccccaagagggcctgtacaacgagctccaaaaggataagatggcagaagcctatagcgagattggtatgaaaggggaacgcagaagaggcaaaggccacgacggactgtaccagggactcagcaccgccaccaaggacacctatgacgctcttcacatgcaggccctgccgcctcgggagggaaggggttctctcctgacctgcggcgatgtggaggagaaccccggacccatgaccaacaagtgtctcctccaaattgctctcctgttgtgcttctccactacagctctttcccaggtgcagctacagcagtcgggcccaggactggtgaagccttcacacaccctgtccctcacctgcactgtctctggtggctccatcagcagtggtggttactactggagttggacccgtcagcacccagggatgggcctggagtggattggatacatctcttacagtgggagtatctattacactccgtccctcaagagtcgacttaccatatcagtggacacgtctaagaaccagttctccctgaagctgagctctgtgactgccgcggacacggccgtatattactgtgcgagtttggattcctggggatctaaccgtgactactggggccagggaaccctggtcaccgtctcgagtggaggtggtggatccgaaattgtgttgacgcagtctccagccaccctgtctttgtctccaggggaaagagccaccctctcctgcagggccagtcagagtgttagcagctacttagcctggtaccaacagaaacctggccaggctcccaggctcctcatctatgatgcatccaacagggccactggcatcccagccaggttcagtggcagtgggtctgggacagacttcactctcaccatcagcagcctagagcctgaagattttgcagtttattactgtcagcagcgtagcaactggccgctcactttcggcggagggaccaaggtggagattaag